European Patent Application EP 4 806 451 A1, published September 16, 2026. Title: BLOCKING AGENT THAT SUPPRESSES VIRUS PROPAGATION, SYNTHETIC NUCLEIC ACID ENCODING BLOCKING AGENT, AND METHOD FOR TREATING AND/OR MITIGATING VIRUS INFECTION BY USING BLOCKING AGENT. Applicant: National Taiwan university. Application US. The sequence listing filed with the application follows.

SEQUENCE LISTING (1 sequence)

SEQ ID NO: 1 - protein, 30 aa, synthetic construct
MVGRNSAIAAGVCGALFIGYCIYFDRKRRS